European Patent Application EP 4 317 169 A1, published February 7, 2024. Title: Method for producing foreign protein using Escherichia coli. Applicant: Kaneka Corporation. The sequence listing filed with the application follows.

SEQUENCE LISTING (54 sequences)

SEQ ID NO: 1 - DNA, 807 bp, Artificial
  Homologous Recombination Donor
ttttttgaattcacaacgtattacctgggaaggttcgcagaaccaggatgcggatgtcagcagcgacggtaaatttatggtaatggtcagctccaatggtgggcagcagcacattgccaaacaagatctggcaacgggaggcgtacaagttctgtcgtccacgttcctggatgaaacgccaagtctggcacctaacggcactatggtaatctacagctcttctcaggggatgggatccgtgctgaatttggtttctacagatgggcgtttcaaagcgcgtcttccggcaactgatggacaggtcaaattccctgcctggtcgccgtatctgtgataataattaattgaatagtaacttcagacatcaactattgagtctgtcgttactggttggtatagcggccccctgggccgcttttgctcaggcaccaatcagtagtgtcggctcaggctcggtcgaagaccgcgtcactcaacttgagcgtatttctaatgctcacagccagcttttaacccaactccagcaacaactttctgataatcaatccgatattgattccctgcgtggtcagattcaggaaaatcagtatcaactgaatcaggtcgtggagcggcaaaagcagatcctgttgcagatcgacagcctcagcagcggtggtgcagcggcgcaatcaaccagcagcgatcaaagcggtgcggcggcatcaacgacgccgacagctgatgctggtactgcgaatgctggcgcgccggtgaaaagcggcgatgcaaacacggattacaatgcagctattggtcgacaaaaaa

SEQ ID NO: 2 - DNA, 840 bp, Artificial
  Homologous Recombination Donor
ttttttgaattccgtgctgaatttggtttctacagatgggcgtttcaaagcgcgtcttccggcaactgatggacaggtcaaattccctgcctggtcgccgtatctgtgataataattaattgaatagtaaaggaatcattgaaatgcaactgaacaaagtgctgaaagggctgatgattgctctgcctgttatggcaattgcggcatgttcttccaacaagaacgccagcaatgacggcagcgaaggcatgctgggtgccctgcagcagaacaacatcgtttacttcgatctggacaagtacgatatccgttctgacttcgctcaaatgctggatgcacatgcaaacttcctgcgtagcaacccgtcttacaaagtcaccgtagaaggtcacgcggacgaacgtggtactccggaatacaacatctccctgggtgaacgtcgtgcgaacgccgttaagatgtacctgcagggtaaaggcgtttctgcagaccagatctccatcgtttcttacggtaaagaaaaacctgcagtactgggtcatgacgaagcggcatactccaaaaaccgtcgtgcggtactggtttactaagagaattgcatgagcagtaacttcagacatcaactattgagtctgtcgttactggttggtatagcggccccctgggccgcttttgctcaggcaccaatcagtagtgtcggctcaggctcggtcgaagaccgcgtcactcaacttgagcgtatttctaatgctcacagccagcttttaacccaactccagcaacaactttctgataatcaatccgatattgattccctgcgtggtcagagtcgacaaaaaa

SEQ ID NO: 3 - DNA, 1066 bp, Artificial
  Homologous Recombination Donor
ttttttgaattcccgcagcttgttaaagagatcacttctactgatgatttctaccgtctgggtaaagaactggctctgcagagcggtctggcacacaaaggtgacgttgtagttatggtttctggtgcactggtaccgagcggcactactaacaccgcatctgttcacgtcctgtaatattgcttttgtgaattaatttgtatatcgaagcgccctgatgggcgctttttttatttaatcgataaccagaagcaataaaaaatcaaatcggatttcactatataatctcactttatctaagatgaatccgatggaagcatcctgttttctctcaatttttttatctaaaacccagcgttcgatgcttctttgagcgaacgatcaaaaataagtgccttcccatcaaaaaaatattctcaacataaaaaactttgtgtaatacttgtaacgctacatggagattaactcaatctagagggtattaataatgaaagctactaaactggtactgggcgcggtaatcctggattctactctgctggcaggttgctccagcaacgctaaaatcgatcagctgtcttctgacgttcagactctgaacgctaaagttgaccagctgagcaacgacgtgaacgcaatgcgttccgacgttcaggctgctaaagatgacgcagctcgtgctaaccagcgtctggacaacatggctactaaataccgcaagtaatagtacctgtgaagtgaaaaatggcgcacattgtgcgccattttttttgtctgccgtttaccgctactgcgtcacgcgtaacatattcccttgctctggttcaccattctgcgctgactctactgaaggcgcattgctggctgcgggagttgctccactgctcaccgaaaccggataccctgcccgacgatacaacgctttatcgactaacttctgatctacagccttattgtctttaaattgcgtaaagcctgctggcagtgtgtatggcattgtctgaacgttctgctgttcttctgccgatagtggtcgatgtacttcaacataacggtcgactttttt

SEQ ID NO: 4 - DNA, 636 bp, Escherichia coli
tatgatgttttcgaagcgacagatggcgcggaaatgcatcagatcctctctgaatatgacatcaacctggtgatcatggatatcaatctgccgggtaagaacggtcttctgttagcgcgtgaactgcgcgagcaggcgaatgttgcgttgatgttcctgactggccgtgacaacgaagtcgataaaattctcggcctcgaaatcggtgcagatgactacatcaccaaaccgttcaacccgcgtgaactgacgattcgtgcacgcaacctactgtcccgtaccatgaatctgggtactgtcagcgaagaacgtcgtagcgttgaaagctacaagttcaatggttgggaactggacatcaacagccgttcgttgatcggccctgatggcgagcagtacaagctgccgcgcagcgagttccgcgccatgcttcacttctgtgaaaacccaggcaaaattcagtcccgtgctgaactgctgaagaaaatgaccggccgtgagctgaaaccgcacgaccgtactgtagacgtgacgatccgccgtattcgtaaacatttcgaatctacgccggatacgccggaaatcatcgccaccattcacggtgaaggttatcgcttctgcggtgatctggaagattaa

SEQ ID NO: 5 - DNA, 81 bp, Escherichia coli
atgcagaccccgcacattcttatcgttgaagacgagttggtaacacgcaacacgttgaaaagtattttcgaagcggaaggc

SEQ ID NO: 6 - DNA, 678 bp, Escherichia coli
tcggggtcaaaggaagaagtacctgataatccgccaaatgaaatttacgcgactgcacaacaaaagctgcaggacggtaactggagacaggcaataacgcaactggaagcgttagataatcgctatccgtttggtccgtattcgcagcaggtgcagctggatctcatctacgcctactataaaaacgccgatttgccgttagcacaggctgccatcgatcgttttattcgccttaacccgacccatccgaatatcgattatgtcatgtacatgcgtggcctgaccaatatggcgctggatgacagtgcgctgcaagggttctttggcgtcgatcgtagcgatcgcgatcctcaacatgcacgagctgcgtttagtgacttttccaaactggtgcgcggctatccgaacagtcagtacaccaccgatgccaccaaacgtctggtattcctgaaagatcgtctggcgaaatatgaatactccgtggccgagtactatacagaacgtggcgcatgggttgccgtcgttaaccgcgtagaaggcatgttgcgcgactacccggatacccaggctacgcgtgatgcgctgccgctgatggaaaatgcataccgtcagatgcagatgaatgcgcaagctgaaaaagtagcgaaaatcatcgccgcaaacagcagcaatacataa

SEQ ID NO: 7 - DNA, 60 bp, Escherichia coli
atgacgcgcatgaaatatctggtggcagccgccacactaagcctgtttttggcgggttgc

SEQ ID NO: 8 - DNA, 876 bp, Escherichia coli
tgtaattctgcgctgttagatcccaaaggacagattggtctggagcaacgttcactgatactgacggcatttggcctgatgttgattgtcgttattcccgcaatcttgatggctgttggtttcgcctggaagtaccgtgcgagcaataaagatgctaagtacagcccgaactggtcacactccaataaagtggaagctgtggtctggacggtacctatcttaatcatcatcttccttgcagtactgacctggaaaaccactcacgctcttgagcctagcaagccgctggcacacgacgagaagcccattaccatcgaagtggtttccatggactggaaatggttcttcatctacccggaacagggcattgctaccgtgaatgaaatcgctttcccggcgaacactccggtgtacttcaaagtgacctccaactccgtgatgaactccttcttcattccgcgtctgggtagccagatttatgccatggccggtatgcagactcgcctgcatctgatcgccaacgaacccggcacttatgacggtatctccgccagctacagcggcccgggcttctcaggcatgaagttcaaagctattgcaacaccggatcgcgccgcattcgaccagtgggtcgcaaaagcgaagcagtcgccgaacaccatgtctgacatggctgcgttcgaaaaactggccgcgcctagcgaatacaaccaggtggaatatttctccaacgtgaaaccagacttgtttgccgatgtaattaacaagtttatggctcacggtaagagcatggacatgacccagccagaaggtgagcacagcgcacacgaaggtatggaaggcatggacatgagccacgcggaatccgcccattaa

SEQ ID NO: 9 - DNA, 72 bp, Escherichia coli
atgagactcaggaaatacaataaaagtttgggatggttgtcattatttgcaggcactgtattgctcagtggc

SEQ ID NO: 10 - DNA, 1524 bp, Escherichia coli
aaaactctggtttattgctcagaaggatctccggaagggtttaacccgcagctgtttacctccggcaccacctatgacgcctcttccgtcccgctttataaccgtctggttgaatttaaaatcggcaccaccgaagtgatcccgggcctcgctgaaaagtgggaagtcagcgaagacggtaaaacctataccttccatctgcgtaaaggtgtgaagtggcacgacaataaagaattcaaaccgacgcgtgaactgaacgccgatgatgtggtgttctcgttcgatcgtcagaaaaacgcgcaaaacccgtaccataaagtttctggcggcagctacgaatacttcgaaggcatgggcttgccagagctgatcagtgaagtgaaaaaggtggacgacaacaccgttcagtttgtgctgactcgcccggaagcgccgttcctcgctgacctggcaatggacttcgcctctattctgtcaaaagaatatgctgatgcgatgatgaaagccggtacaccggaaaaactggacctcaacccaatcggaaccggtccgttccagttacagcagtatcaaaaagattcccgtatccgctacaaagcgtttgatggctactggggcaccaaaccgcagatcgatacgctggttttctctattacccctgacgcttccgtgcgttacgcgaaattgcagaagaatgaatgccaggtgatgccgtacccgaacccggcagatatcgctcgcatgaagcaggataaatccatcaatctgatggaaatgccggggctgaacgtcggttatctctcgtataacgtgcagaaaaaaccactcgatgacgtgaaagttcgccaggctctgacctacgcggtgaacaaagacgcgatcatcaaagcggtttatcagggcgcgggcgtatcagcgaaaaacctgatcccgccaaccatgtggggctataacgacgacgttcaggactacacctacgatcctgaaaaagcgaaagccttgctgaaagaagcgggtctggaaaaaggtttctccatcgacctgtgggcgatgccggtacaacgtccgtataacccgaacgctcgccgcatggcggagatgattcaggcagactgggcgaaagtcggcgtgcaggccaaaattgtcacctacgaatggggtgagtacctcaagcgtgcgaaagatggcgagcaccagacggtaatgatgggctggactggcgataacggggatccggataacttcttcgccaccctgttcagctgcgccgcctctgaacaaggctccaactactcaaaatggtgctacaaaccgtttgaagatctgattcaaccggcgcgtgctaccgacgaccacaataaacgcgttgaactgtacaaacaagcgcaggtggtgatgcacgatcaggctccggcactgatcatcgctcactccaccgtgtttgaaccggtacgtaaagaagttaaaggctatgtggttgatccattaggcaaacatcacttcgaaaacgtctctatcgaataa

SEQ ID NO: 11 - DNA, 84 bp, Escherichia coli
atgcgtatttccttgaaaaagtcagggatgctgaagcttggtctcagcctggtggctatgaccgtcgcagcaagtgttcaggct

SEQ ID NO: 12 - DNA, 84 bp, Escherichia coli
tgcaacaccacgcgtggcgttggtgaagacatttctgatggcggtaacgcgatttctggcgcagcaacgaaagcgcagcaataa

SEQ ID NO: 13 - DNA, 63 bp, Escherichia coli
atggtgaagaagacaattgcagcgatcttttctgttctggtgctttcaacagtattaactgcc

SEQ ID NO: 14 - DNA, 162 bp, Escherichia coli
aaaatcgatcagctgtcttctgacgttcagactctgaacgctaaagttgaccagctgagcaacgacgtgaacgcaatgcgttccgacgttcaggctgctaaagatgacgcagctcgtgctaaccagcgtctggacaacatggctactaaataccgcaagtaa

SEQ ID NO: 15 - DNA, 75 bp, Escherichia coli
atgaaagctactaaactggtactgggcgcggtaatcctgggttctactctgctggcaggttgctccagcaacgct

SEQ ID NO: 16 - DNA, 489 bp, Escherichia coli
tgtagtgcaaataacaccgcaaagaatatgcatcctgagacacgtgcagtgggtagtgaaacatcatcactgcaagcttctcaggatgaatttgaaaacctggttcgtaatgtcgacgtaaaatcgcgaattatggatcagtatgctgactggaaaggcgtacgttatcgtctgggcggcagcactaaaaaaggtatcgattgttctggtttcgtacagcgtacattccgtgagcaatttggcttagaacttccgcgttcgacttacgaacagcaggaaatgggtaaatctgtttcccgcagtaatttgcgtacgggtgatttagttctgttccgtgccggttcaacgggacgccatgtcggtatttatatcggcaacaatcagtttgtccatgcttccaccagcagtggtgttattatttccagcatgaatgaaccgtactggaagaagcgttacaacgaagcacgccgggttctcagccgcagctaa

SEQ ID NO: 17 - DNA, 78 bp, Escherichia coli
atggtcaaatctcaaccgattttgagatatatcttgcgcgggattcccgcgattgcagtagcggttctgctttctgca

SEQ ID NO: 18 - DNA, 2496 bp, Escherichia coli
ggctcgatttatggcctataccgctacatcgagccacaactgccggatgtggcgacattaaaagatgttcgcctgcaaattccgatgcagatttacagcgccgatggcgagctgattgctcaatacggtgagaaacgtcgtattccggttacgttggatcaaatcccaccggagatggtgaaagcctttatcgcgacagaagacagccgcttctacgagcatcacggcgttgacccggtggggatcttccgtgcagcaagcgtggcgctgttctccggtcacgcgtcacaaggggcaagtaccattacccagcagctggcgagaaacttcttcctcagtccagaacgcacgctgatgcgtaagattaaggaagtcttcctcgcgattcgcattgaacagctgctgacgaaagacgagatcctcgagctttatctgaacaagatttaccttggttaccgcgcctatggtgtcggtgctgcggcacaagtctatttcggaaaaacggtcgaccaactgacgctgaacgaaatggcggtgatagccgggctgccgaaagcgccttccaccttcaacccgctctactcgatggatcgtgccgtcgcgcggcgtaacgtcgtgctgtcgcggatgctggatgaagggtatatcacccaacaacagttcgatcagacacgcactgaggcgattaacgctaactatcacgcgccggagattgctttctctgcgccgtacctgagcgaaatggtgcgccaggagatgtataaccgttatggcgaaagtgcctatgaagacggttatcgcatttacaccaccatcacccgcaaagtgcagcaggccgcgcagcaggcggtacgtaataacgtgctggactacgacatgcgccacggctatcgcggcccggcaaatgtgctgtggaaagtgggcgagtcggcgtgggataacaacaagattaccgatacgctgaaggcgctgccaacctatggtccgctgctgcctgccgcagtcaccagcgccaatcctcagcaagcgacggcgatgctggcggacgggtcgaccgtcgcattgagtatggaaggcgttcgctgggcgcgtccttaccgttcggatactcagcaaggaccgacgccgcgtaaagtgaccgatgttctgcaaacgggtcagcaaatctgggttcgtcaggttggcgatgcatggtggctggcacaagtgccggaagtgaactcggcgctggtgtcgatcaatccgcaaaacggtgccgttatggcgctggtcggtggctttgatttcaatcagagcaagtttaaccgcgccacccaggcactgcgtcaggtgggttccaacatcaaaccgttcctctacaccgcggcgatggataaaggtctgacgctggcaagtatgttgaacgatgtgccaatttctcgctgggatgcaagtgccggttctgactggcagccgaagaactcaccaccgcagtatgctggtccaattcgcttacgtcaggggctgggtcagtcgaaaaacgtggtgatggtacgcgcaatgcgggcgatgggcgtcgactacgctgcagaatatctgcaacgcttcggcttcccggcacaaaacattgtccacaccgaatcgctggcgctgggttcagcgtccttcaccccaatgcaggtggcgcgcggctacgcggtcatggcgaacggcggcttcctggtggacccgtggtttatcagcaaaattgaaaacgatcagggcggcgtgattttcgaagcgaaaccgaaagtagcctgcccggaatgcgatattccggtgatttacggtgatacgcagaaatcgaacgtgctggaaaataacgatgttgaagatgtcgctatctcccgcgagcagcagaatgtttctgtaccaatgccgcagctggagcaggcaaatcaggcgttagtggcgaagactggcgcgcaggagtacgcaccgcacgtcatcaacactccgctggcattcctgattaagagtgctttgaacaccaatatctttggtgagccaggctggcagggtactggctggcgtgcaggtcgtgatttgcagcgtcgcgatatcggcgggaaaaccgggaccactaacagttcgaaagatgcgtggttctcgggttacggtccgggcgttgtgacctcggtctggattggctttgatgatcaccgtcgtaatctcggtcatacaacggcttccggagcgattaaagatcagatctcaggttacgaaggcggtgccaagagtgcccagcctgcatgggacgcttatatgaaagccgttcttgaaggtgtgccggagcagccgctgacgccgccaccgggtattgtgacggtgaatatcgatcgcagcaccgggcagttagctaatggtggcaacagccgcgaagagtatttcatcgaaggtacgcagccgacacaacaggcagtgcacgaggtgggaacgaccattatcgataatggcgaggcacaggaattgttctga

SEQ ID NO: 19 - DNA, 57 bp, Escherichia coli
gtgaagttcgtaaagtattttttgatccttgcagtctgttgcattctgctgggagca

SEQ ID NO: 20 - DNA, 2496 bp, Escherichia coli
aaaccgacgcgtccggtcaaacaaaaggtaagccgtcgtcgttacgaagatgacgatgattacgacgattatgatgactatgaggatgaagaaccgatgccgcgcaaaggtaagggcaaaggcaaagggcgtaagcctcgtggcaaacgcggctggctatggctactgctaaaactggctatcgtttttgccgtgctgatcgccatttacggcgtttatctcgatcaaaaaattcgtagccgtattgatggcaaggtctggcaactgcctgcggcagtttatggccgaatggtcaatcttgagccagacatgaccatcagcaagaacgagatggtgaagctgctggaggcgacccagtatcgtcaggtgtcgaaaatgacccgtcctggcgaatttaccgtgcaggccaacagcattgagatgattcgccgtccgtttgatttcccggacagtaaagaaggacaggtgcgcgcgcgtctgacctttgatggcgatcatctggcgacgatcgtcaatatggagaacaaccgtcagttcggtttcttccgtcttgatccgcgtctgatcaccatgatctcttcgccaaacggtgagcagcgtctgtttgtgccgcgcagtggtttcccggatttgctggtggatactttgctggcgacagaagaccgtcatttttacgagcatgatggaatcagtctctactcaatcggacgtgcggtgctggcaaacctgaccgccggacgcacggtacagggtgcgagtacgctgacgcaacagctggtgaaaaacctgttcctctccagcgagcgttcttactggcgtaaagcgaacgaagcttacatggcgctgatcatggacgcgcgttacagcaaagaccgtattcttgagctgtatatgaacgaggtgtatctcggtcagagcggcgacaacgaaatccgcggcttcccgctggcaagcttgtattactttggtcgcccggtagaagagctaagcctcgaccagcaggcgctgttagtcggtatggtgaaaggggcgtccatctacaacccgtggcgtaacccaaaactggcgctggagcgacgtaatctggtgctgcgtctgctgcaacagcaacagattattgatcaagaactctatgacatgttgagtgcccgtccgctgggggttcagccgcgcggtggggtgatctctcctcagccagcctttatgcaactggtgcgtcaggagctgcaggcaaaactgggcgataaggtaaaagatctctccggcgtgaagatcttcactacctttgactcggtggcccaggacgcggcagaaaaagccgccgtggaaggcattccggcactgaagaaacagcgtaagttgagcgatcttgaaactgcgattgtggtcgtcgaccgctttagtggtgaagttcgtgcgatggtcggaggttctgagccgcagtttgcgggctacaaccgtgcgatgcaggcgcgtcgttcgattggttcccttgcaaaaccagcgacttatctgacggccttaagccagccgaaaatctatcgtctgaatacgtggattgcggatgcgccaattgcgctgcgtcagccgaatggccaggtctggtcaccgcagaatgatgaccgtcgttatagcgaaagcggcagagtgatgctggtggatgcgttgacccgttcgatgaacgtgccgacggtaaatctggggatggcgctggggctgcctgcggttacggagacctggattaaactgggcgtaccgaaagatcagttgcatccggttccggcaatgctgctgggggcgttgaacttaacgccaatcgaagtggcgcaggcattccagaccatcgccagcggtggtaaccgtgcaccgctttctgcgctgcgttcggtaatcgcggaagatggcaaagtgctgtatcagagcttcccgcaggcggaacgcgctgttccggcgcaggcggcgtatctgacactatggaccatgcagcaggtggtacaacgcggtacgggtcgtcagcttggggcgaaatacccgaacctgcatctggcagggaaaacagggactaccaacaataacgtagatacctggtttgcgggcattgacggcagcacggtgaccatcacctgggtcggccgtgataacaaccagccgaccaaactgtatggtgccagcggggcaatgtcgatttatcagcgttatctggctaaccagacgccaacgccgctgaatcttgttccgccagaagatattgcagatatgggcgtggactacgacggcaactttgtttgcagcggtggcatgcgtatcttgccggtctggaccagcgatccgcaatcgctgtgccagcagagcgagatgcagcagcagccgtcaggcaatccgtttgatcagtcttctcagccgcagcaacagccgcaacagcaacctgctcagcaagagcagaaagacagcgacggtgtagccggttggatcaaggatatgtttggtagtaattaa

SEQ ID NO: 21 - DNA, 39 bp, Escherichia coli
atggccgggaatgaccgcgagccaattggacgcaaaggg

SEQ ID NO: 22 - DNA, 846 bp, Escherichia coli
cttacgcttgcaggatgcagtaatacttcctggcgtaaaagtgaagtcctcgcggtaccattgcaaccgactttacagcaggaagtgattctggcacgtatggaacaaatccttgccagtcgggctttaaccgatgacgaacgcgcacagcttttatatgagcgcggagtgttgtatgatagtctcggtctgagggcattagcgcgtaacgatttttcgcaagcgctggcaatccgaccggatatgcctgaagtattcaattacttaggcatatatttaacgcaggcaggcaattttgatgctgcctatgaagcgtttgattctgtacttgagcttgatccaacttacaactacgcgcacttgaatcgcgggatcgcattatattacggcggtcgtgacaagttagcgcaagatgatctgctggcgttttatcaagacgatcccaatgatcctttccgtagtctgtggctttatctcgccgagcagaagctcgatgagaagcaggctaaagaagtgttgaaacagcacttcgaaaaatcggataaggaacagtggggatggaacattgtcgagttctacctgggcaacattagcgaacaaacgttaatggaaaggctcaaggcggacgcaacggataacacctcgctcgctgagcatctcagtgaaaccaacttctatttaggtaagtactacctaagtctgggggatttggacagcgccacggcactgttcaaactggcggttgccaacaacgttcataactttgttgagcaccgatacgcattgttggaattatcgctcctgggccaggaccaagatgacctggcagaatcggaccagcaatag

SEQ ID NO: 23 - DNA, 39 bp, Escherichia coli
atgaagccttttttgcgctggtgtttcgttgcgacagca

SEQ ID NO: 24 - DNA, 978 bp, Escherichia coli
gctccgaaagataacacctggtacactggtgctaaactgggctggtcccagtaccatgacactggtttcatcaacaacaatggcccgacccatgaaaaccaactgggcgctggtgcttttggtggttaccaggttaacccgtatgttggctttgaaatgggttacgactggttaggtcgtatgccgtacaaaggcagcgttgaaaacggtgcatacaaagctcagggcgttcaactgaccgctaaactgggttacccaatcactgacgacctggacatctacactcgtctgggtggcatggtatggcgtgcagacactaaatccaacgtttatggtaaaaaccacgacaccggcgtttctccggtcttcgctggcggtgttgagtacgcgatcactcctgaaatcgctacccgtctggaataccagtggaccaacaacatcggtgacgcacacaccatcggcactcgtccggacaacggcatgctgagcctgggtgtttcctaccgtttcggtcagggcgaagcagctccagtagttgctccggctccagctccggcaccggaagtacagaccaagcacttcactctgaagtctgacgttctgttcaacttcaacaaagcaaccctgaaaccggaaggtcaggctgctctggatcagctgtacagccagctgagcaacctggatccgaaagacggttccgtagttgttctgggttacaccgaccgcatcggttctgacgcttacaaccagggtctgtccgagcgccgtgctcagtctgttgttgattacctgatctccaaaggtatcccggcagacaagatctccgcacgtggtatgggcgaatccaacccggttactggcaacacctgtgacaacgtgaaacagcgtgctgcactgatcgactgcctggctccggatcgtcgcgtagagatcgaagttaaaggtatcaaagacgttgtaactcagccgcaggcttaa

SEQ ID NO: 25 - DNA, 63 bp, Escherichia coli
atgaaaaagacagctatcgcgattgcagtggcactggctggtttcgctaccgtagcgcaggcc

SEQ ID NO: 26 - DNA, 1554 bp, Escherichia coli
gctgatgtacccgcaggcgtcacactggcggaaaaacaaacactggtacgtaacaatggttcagaagttcagtcattagatccgcacaaaattgaaggtgttccggagtctaatatcagccgagacctgtttgaaggcttactggtcagcgatcttgacggtcatccagcacctggcgtcgctgaatcctgggataataaagacgcgaaagtctggaccttccatttgcgtaaagatgcgaaatggtctgatggcacgccagtcacagcacaagactttgtgtatagctggcaacgttctgttgatccgaacactgcttctccgtatgccagttatctgcaatatgggcatatcgccggtattgatgaaattcttgaagggaaaaaaccgattaccgatctcggcgtgaaagctattgatgatcacacattagaagtcaccttaagtgaacccgttccgtacttctataaattacttgttcacccatcaacttcaccggtgccaaaagccgctatcgagaaattcggcgaaaaatggacccagcctggtaatatcgtcaccaacggtgcctataccttaaaagattgggtcgtaaacgaacgaatcgttcttgaacgcagcccgacctactggaacaacgcgaaaaccgttattaaccaggtaacctatttgcctattgcttctgaagttaccgatgtcaaccgctaccgtagtggtgaaatcgacatgacgaataacagcatgccgatcgaattgttccagaagctgaaaaaagagatcccggacgaagttcacgttgatccatacctgtgcacttactattacgaaattaacaaccagaaaccgccattcaacgatgtgcgtgtgcgtaccgcactgaaactaggtatggaccgcgatatcattgttaataaagtgaaagcgcagggcaacatgcccgcctatggttacactccaccgtatactgatggcgcaaaattgactcagccagaatggtttggctggagccaggaaaaacgtaacgaagaagcgaaaaaactgctggctgaagcgggttataccgcagacaaaccgttgaccatcaacctgttgtataacacctccgatctgcataaaaagctggcgattgctgcctcttcattgtggaagaaaaacattggtgtaaacgtcaaactggttaaccaggagtggaaaacgttcctcgacacccgtcaccagggtacttttgatgtggcccgtgcaggctggtgtgctgactacaacgaaccaacttccttcctgaacaccatgctttcgaacagctcgatgaataccgcgcattataagagcccggcctttgacagcattatggcggaaacgctgaaagtgactgacgaggcgcagcgcacagctctgtacactaaagcagaacaacagctggataaggattcggccattgttcctgtttattactacgtgaatgcgcgtctggtgaaaccgtgggttggtggctataccggcaaagatccgctggataatacctatacccggaatatgtacattgtgaagcactaa

SEQ ID NO: 27 - DNA, 78 bp, Escherichia coli
atgaccaacatcaccaagagaagtttagtagcagctggcgttctggctgcgctaatggcagggaatgtcgcgctggca

SEQ ID NO: 28 - DNA, 459 bp, Escherichia coli
tgttcttccaacaagaacgccagcaatgacggcagcgaaggcatgctgggtgccggcactggtatggatgcgaacggcggcaacggcaacatgtcttccgaagagcaggctcgtctgcaaatgcaacagctgcagcagaacaacatcgtttacttcgatctggacaagtacgatatccgttctgacttcgctcaaatgctggatgcacatgcaaacttcctgcgtagcaacccgtcttacaaagtcaccgtagaaggtcacgcggacgaacgtggtactccggaatacaacatctccctgggtgaacgtcgtgcgaacgccgttaagatgtacctgcagggtaaaggcgtttctgcagaccagatctccatcgtttcttacggtaaagaaaaacctgcagtactgggtcatgacgaagcggcatactccaaaaaccgtcgtgcggtactggtttactaa

SEQ ID NO: 29 - DNA, 63 bp, Escherichia coli
atgcaactgaacaaagtgctgaaagggctgatgattgctctgcctgttatggcaattgcggca

SEQ ID NO: 30 - DNA, 417 bp, Escherichia coli
tgtgttaataacgacaccctgtcaggggatgtttataccgcttctgaagcgaaacaagtacagaatgtcagctatggcaccatcgttaacgtacgtccggtacagattcagggcggtgatgattccaacgttatcggtgcaattggcggtgctgttcttggtggtttcctggggaatactgttggtggcggaaccgggcgttctctggctactgcagcaggcgctgttgcaggtggcgtagctggtcagggcgtacagagtgcaatgaacaaaacgcagggtgtcgagctggaaattcgtaaagacgatggtaataccatcatggtggtacagaaacaaggcaacactcgtttctctccgggccaacgtgtcgtactggccagcaatggcagtcaggtgaccgtttctccgcgctaa

SEQ ID NO: 31 - DNA, 51 bp, Escherichia coli
atgattaaacgcgtattggttgtttcaatggtaggtctgtctcttgtcggt

SEQ ID NO: 32 - DNA, 1266 bp, Escherichia coli
gtgtcaaaggcaaccgaacaaaacgacaagctcaagcgggcgataattatttcagcagtgctgcatgtcatcttatttgcggcgctgatctggagttcgttcgatgagaatatagaagcttcagccggaggcggcggtggttcgtccatcgacgctgtcatggttgattcaggtgcggtagttgagcagtacaaacgcatgcaaagccaggaatcaagcgcgaagcgttctgatgaacagcgcaagatgaaggaacagcaggctgctgaagaactgcgtgagaaacaagcggctgaacaggaacgcctgaagcaacttgagaaagagcggttagcggctcaggagcagaaaaagcaggctgaagaagccgcaaaacaggccgagttaaagcagaagcaagctgaagaggcggcagcgaaagcggcggcagatgctaaagcgaaggccgaagcagatgctaaagctgcggaagaagcagcgaagaaagcggctgcagacgcaaagaaaaaagcagaagcagaagccgccaaagccgcagccgaagcgcagaaaaaagccgaggcagccgctgcggcactgaagaagaaagcggaagcggcagaagcagctgcagctgaagcaagaaagaaagcggcaactgaagctgctgaaaaagccaaagcagaagctgagaagaaagcggctgctgaaaaggctgcagctgataagaaagcggcagcagagaaagctgcagccgacaaaaaagcagcagaaaaagcggctgctgaaaaggcagcagctgataagaaagcagcggcagaaaaagccgccgcagacaaaaaagcggcagcggcaaaagctgcagctgaaaaagccgctgcagcaaaagcggccgcagaggcagatgatattttcggtgagctaagctctggtaagaatgcaccgaaaacggggggaggggcgaaagggaacaatgcttcgcctgccgggagtggtaatactaaaaacaatggcgcatcaggggccgatatcaataactatgccgggcagattaaatctgctatcgaaagtaagttctatgacgcatcgtcctatgcaggcaaaacctgtacgctgcgcataaaactggcacccgatggtatgttactggatatcaaacctgaaggtggcgatcccgcactttgtcaggctgcgttggcagcagctaaacttgcgaagatcccgaaaccaccaagccaggcagtatatgaagtgttcaaaaacgcgccattggacttcaaaccgtaa

SEQ ID NO: 33 - protein, 152 aa, Escherichia coli
CSSNKNASNDGSEGMLGAGTGMDANGGNGNMSSEEQARLQMQQLQQNNIVYFDLDKYDIRSDFAQMLDAHANFLRSNPSYKVTVEGHADERGTPEYNISLGERRANAVKMYLQGKGVSADQISIVSYGKEKPAVLGHDEAAYSKNRRAVLVY

SEQ ID NO: 34 - protein, 21 aa, Escherichia coli
MQLNKVLKGLMIALPVMAIAA

SEQ ID NO: 35 - protein, 137 aa, Escherichia coli
CSAGTGMDANGGNGNMSSEEQARLQMQQLQQNNIVYFDLDKYDIRSDFAQMLDAHANFLRSNPSYKVTVEGHADERGTPEYNISLGERRANAVKMYLQGKGVSADQISIVSYGKEKPAVLGHDEAAYSKNRRAVLVY

SEQ ID NO: 36 - DNA, 414 bp, Escherichia coli
tgttctgccggcactggtatggatgcgaacggcggcaacggcaacatgtcttccgaagagcaggctcgtctgcaaatgcaacagctgcagcagaacaacatcgtttacttcgatctggacaagtacgatatccgttctgacttcgctcaaatgctggatgcacatgcaaacttcctgcgtagcaacccgtcttacaaagtcaccgtagaaggtcacgcggacgaacgtggtactccggaatacaacatctccctgggtgaacgtcgtgcgaacgccgttaagatgtacctgcagggtaaaggcgtttctgcagaccagatctccatcgtttcttacggtaaagaaaaacctgcagtactgggtcatgacgaagcggcatactccaaaaaccgtcgtgcggtactggtttactaa

SEQ ID NO: 37 - protein, 127 aa, Escherichia coli
CSSNKNASNDGSEGMLGALQQNNIVYFDLDKYDIRSDFAQMLDAHANFLRSNPSYKVTVEGHADERGTPEYNISLGERRANAVKMYLQGKGVSADQISIVSYGKEKPAVLGHDEAAYSKNRRAVLVY

SEQ ID NO: 38 - DNA, 384 bp, Escherichia coli
tgttcttccaacaagaacgccagcaatgacggcagcgaaggcatgctgggtgccctgcagcagaacaacatcgtttacttcgatctggacaagtacgatatccgttctgacttcgctcaaatgctggatgcacatgcaaacttcctgcgtagcaacccgtcttacaaagtcaccgtagaaggtcacgcggacgaacgtggtactccggaatacaacatctccctgggtgaacgtcgtgcgaacgccgttaagatgtacctgcagggtaaaggcgtttctgcagaccagatctccatcgtttcttacggtaaagaaaaacctgcagtactgggtcatgacgaagcggcatactccaaaaaccgtcgtgcggtactggtttactaa

SEQ ID NO: 39 - protein, 133 aa, Escherichia coli
CSSNKNASNDGSEGMLGAGTGMDANGGNGNMSSEEQARLQMQQFAQMLDAHANFLRSNPSYKVTVEGHADERGTPEYNISLGERRANAVKMYLQGKGVSADQISIVSYGKEKPAVLGHDEAAYSKNRRAVLVY

SEQ ID NO: 40 - DNA, 402 bp, Escherichia coli
tgttcttccaacaagaacgccagcaatgacggcagcgaaggcatgctgggtgccggcactggtatggatgcgaacggcggcaacggcaacatgtcttccgaagagcaggctcgtctgcaaatgcaacagttcgctcaaatgctggatgcacatgcaaacttcctgcgtagcaacccgtcttacaaagtcaccgtagaaggtcacgcggacgaacgtggtactccggaatacaacatctccctgggtgaacgtcgtgcgaacgccgttaagatgtacctgcagggtaaaggcgtttctgcagaccagatctccatcgtttcttacggtaaagaaaaacctgcagtactgggtcatgacgaagcggcatactccaaaaaccgtcgtgcggtactggtttactaa

SEQ ID NO: 41 - protein, 120 aa, Escherichia coli
CSSNKNASNDGSEGMLGAGTGMDANGGNGNMSSEEQARLQMQQLQQNNIVYFDLDKYDIRSPEYNISLGERRANAVKMYLQGKGVSADQISIVSYGKEKPAVLGHDEAAYSKNRRAVLVY

SEQ ID NO: 42 - DNA, 363 bp, Escherichia coli
tgttcttccaacaagaacgccagcaatgacggcagcgaaggcatgctgggtgccggcactggtatggatgcgaacggcggcaacggcaacatgtcttccgaagagcaggctcgtctgcaaatgcaacagctgcagcagaacaacatcgtttacttcgatctggacaagtacgatatccgttctccggaatacaacatctccctgggtgaacgtcgtgcgaacgccgttaagatgtacctgcagggtaaaggcgtttctgcagaccagatctccatcgtttcttacggtaaagaaaaacctgcagtactgggtcatgacgaagcggcatactccaaaaaccgtcgtgcggtactggtttactaa

SEQ ID NO: 43 - protein, 124 aa, Escherichia coli
CSSNKNASNDGSEGMLGAGTGMDANGGNGNMSSEEQARLQMQQLQQNNIVYFDLDKYDIRSDFAQMLDAHANFLRSNPSYKVTVEGHADERGTISIVSYGKEKPAVLGHDEAAYSKNRRAVLVY

SEQ ID NO: 44 - DNA, 375 bp, Escherichia coli
tgttcttccaacaagaacgccagcaatgacggcagcgaaggcatgctgggtgccggcactggtatggatgcgaacggcggcaacggcaacatgtcttccgaagagcaggctcgtctgcaaatgcaacagctgcagcagaacaacatcgtttacttcgatctggacaagtacgatatccgttctgacttcgctcaaatgctggatgcacatgcaaacttcctgcgtagcaacccgtcttacaaagtcaccgtagaaggtcacgcggacgaacgtggtactatctccatcgtttcttacggtaaagaaaaacctgcagtactgggtcatgacgaagcggcatactccaaaaaccgtcgtgcggtactggtttactaa

SEQ ID NO: 45 - protein, 122 aa, Escherichia coli
CSSNKNASNDGSEGMLGAGTGMDANGGNGNMSSEEQARLQMQQLQQNNIVYFDLDKYDIRSDFAQMLDAHANFLRSNPSYKVTVEGHADERGTPEYNISLGERRANAVKMYLQGKGVSADQI

SEQ ID NO: 46 - DNA, 369 bp, Escherichia coli
tgttcttccaacaagaacgccagcaatgacggcagcgaaggcatgctgggtgccggcactggtatggatgcgaacggcggcaacggcaacatgtcttccgaagagcaggctcgtctgcaaatgcaacagctgcagcagaacaacatcgtttacttcgatctggacaagtacgatatccgttctgacttcgctcaaatgctggatgcacatgcaaacttcctgcgtagcaacccgtcttacaaagtcaccgtagaaggtcacgcggacgaacgtggtactccggaatacaacatctccctgggtgaacgtcgtgcgaacgccgttaagatgtacctgcagggtaaaggcgtttctgcagaccagatctaa

SEQ ID NO: 47 - protein, 148 aa, Escherichia coli
CSSNKNASNDGSEGMLGAGTGMDANGGNGNMSSEEQARLQMQQLQQNNIVYFDLDKYDIRSDFAQMLDAHANFLRSNPSYKVTVEGHADERGTPEYNISLGERRANAVKMYLQGKGVSADQISIVEKPAVLGHDEAAYSKNRRAVLVY

SEQ ID NO: 48 - DNA, 447 bp, Escherichia coli
tgttcttccaacaagaacgccagcaatgacggcagcgaaggcatgctgggtgccggcactggtatggatgcgaacggcggcaacggcaacatgtcttccgaagagcaggctcgtctgcaaatgcaacagctgcagcagaacaacatcgtttacttcgatctggacaagtacgatatccgttctgacttcgctcaaatgctggatgcacatgcaaacttcctgcgtagcaacccgtcttacaaagtcaccgtagaaggtcacgcggacgaacgtggtactccggaatacaacatctccctgggtgaacgtcgtgcgaacgccgttaagatgtacctgcagggtaaaggcgtttctgcagaccagatctccatcgttgaaaaacctgcagtactgggtcatgacgaagcggcatactccaaaaaccgtcgtgcggtactggtttactaa

SEQ ID NO: 49 - protein, 148 aa, Escherichia coli
CSSNKNASNDGSEGMLGAGTGMDANGGNGNMSSEEQARLQMQQLQQNNIVYFDLDKYDIRSDFAQMLDAHANFLRSNPSYKVTVEGHADERGTPEYNISLGERRANAVKMYLQGKGVSADQISIVSYGKEKPAVLGHDEAAYSAVLVY

SEQ ID NO: 50 - DNA, 447 bp, Escherichia coli
tgttcttccaacaagaacgccagcaatgacggcagcgaaggcatgctgggtgccggcactggtatggatgcgaacggcggcaacggcaacatgtcttccgaagagcaggctcgtctgcaaatgcaacagctgcagcagaacaacatcgtttacttcgatctggacaagtacgatatccgttctgacttcgctcaaatgctggatgcacatgcaaacttcctgcgtagcaacccgtcttacaaagtcaccgtagaaggtcacgcggacgaacgtggtactccggaatacaacatctccctgggtgaacgtcgtgcgaacgccgttaagatgtacctgcagggtaaaggcgtttctgcagaccagatctccatcgtttcttacggtaaagaaaaacctgcagtactgggtcatgacgaagcggcatactccgcggtactggtttactaa

SEQ ID NO: 51 - protein, 78 aa, Escherichia coli
MKATKLVLGAVILGSTLLAGCSSNAKIDQLSSDVQTLNAKVDQLSNDVNAMRSDVQAAKDDAARANQRLDNMATKYRK

SEQ ID NO: 52 - protein, 346 aa, Escherichia coli
MKKTAIAIAVALAGFATVAQAAPKDNTWYTGAKLGWSQYHDTGFINNNGPTHENQLGAGAFGGYQVNPYVGFEMGYDWLGRMPYKGSVENGAYKAQGVQLTAKLGYPITDDLDIYTRLGGMVWRADTKSNVYGKNHDTGVSPVFAGGVEYAITPEIATRLEYQWTNNIGDAHTIGTRPDNGMLSLGVSYRFGQGEAAPVVAPAPAPAPEVQTKHFTLKSDVLFNFNKATLKPEGQAALDQLYSQLSNLDPKDGSVVVLGYTDRIGSDAYNQGLSERRAQSVVDYLISKGIPADKISARGMGESNPVTGNTCDNVKQRAALIDCLAPDRRVEIEVKGIKDVVTQPQA

SEQ ID NO: 53 - protein, 421 aa, Escherichia coli
MSKATEQNDKLKRAIIISAVLHVILFAALIWSSFDENIEASAGGGGGSSIDAVMVDSGAVVEQYKRMQSQESSAKRSDEQRKMKEQQAAEELREKQAAEQERLKQLEKERLAAQEQKKQAEEAAKQAELKQKQAEEAAAKAAADAKAKAEADAKAAEEAAKKAAADAKKKAEAEAAKAAAEAQKKAEAAAAALKKKAEAAEAAAAEARKKAATEAAEKAKAEAEKKAAAEKAAADKKAAAEKAAADKKAAEKAAAEKAAADKKAAAEKAAADKKAAAAKAAAEKAAAAKAAAEADDIFGELSSGKNAPKTGGGAKGNNASPAGSGNTKNNGASGADINNYAGQIKSAIESKFYDASSYAGKTCTLRIKLAPDGMLLDIKPEGGDPALCQAALAAAKLAKIPKPPSQAVYEVFKNAPLDFKP

SEQ ID NO: 54 - DNA, 780 bp, Artificial
  anti vWF VHH antibody
gaagtgcagttagtggagagtggcggcggtctggtgcagccaggtggttctctgcgcctgagctgtgcggcttccggccgtaccttctcgtacaaccctatgggctggtttcggcaggcaccgggaaaagggcgcgaacttgtggctgcgattagccgtacgggcggaagcacctattatccggactccgttgaagggcgctttaccatttcccgcgacaatgccaaacgcatggtatatctccagatgaacagtttacgggcagaagatacggcggtttactattgcgccgctgccggtgttcgtgcagaggatggtcgcgtgcgtacacttccatcggagtacactttctggggtcaaggcactcaagtcaccgtcagttcggcggccgcggaagttcagctcgttgaaagcggcggtgggctggtacagcctggcggatctctgcgtctgtcttgtgccgcaagtggccgcaccttcagctataatccgatggggtggtttcgccaagcgccgggtaaaggtcgtgaactggtggctgccatctcacgtacaggcggctctacctactatcccgactcagtggagggtcgctttacgatcagccgcgataatgcgaaacgtatggtctacttgcaaatgaactccttacgcgccgaagatacagcggtctattactgcgctgccgctggtgtgcgcgcggaagatgggcgtgttcgcacgctgccgtcggaatatacgttttggggccagggcacccaggtaaccgtcagctcataa